European Patent Application EP 4 375 300 A1, published May 29, 2024. Title: 药物组合物及用途. Applicant: 中山康方生物医药有限公司. The sequence listing filed with the application follows.

SEQUENCE LISTING (78 sequences)

SEQ ID NO: 1 - protein, 121 aa, synthetic construct
EVQLQESGPGLVKPSQSLSLTCTVTGHSFTSDYAWNWIRQFPGNRLEWMGYISYSDSTNYNPSLKSRISITRDTSKNQFFLQMNSVTTEDTATYYCARLDYGNYGGAMDYWGQGTSVTVSS

SEQ ID NO: 2 - DNA, 363 bp, synthetic construct
  source 1..363: mol_type = other DNA
gaggtgcagctgcaggagtctggacctggcctggtgaaaccctctcagtctctgtccctcacctgcactgtcactggccactcattcaccagtgattatgcctggaactggatccggcagtttccaggaaacagactggagtggatgggctacataagctacagtgatagcactaactacaacccatctctcaaaagtcgaatctctatcactcgagacacatccaagaaccagttcttcttgcagatgaattctgtgactactgaggacacagccacatattactgtgcaagattggactatggtaactacggtggggctatggactactggggtcaagggacctcagtcaccgtctcctca

SEQ ID NO: 3 - protein, 9 aa, synthetic construct
GHSFTSDYA

SEQ ID NO: 4 - protein, 7 aa, synthetic construct
ISYSDST

SEQ ID NO: 5 - protein, 14 aa, synthetic construct
ARLDYGNYGGAMDY

SEQ ID NO: 6 - protein, 107 aa, synthetic construct
DIVLTQSHEFMSTSLRDRVSITCKSSQHVSTAVAWYQQKPGQSPKLLIYSASYRYTGVPDRFTGSGSGTDFTFTISSVKAEDLAVYYCQQHYITPWTFGGGTKLEIK

SEQ ID NO: 7 - DNA, 321 bp, synthetic construct
  source 1..321: mol_type = other DNA
gatattgtgctaactcagtctcacgaattcatgtccacctcattacgagacagggtcagcatcacctgcaaatccagtcaacatgtgagtactgctgtagcctggtatcaacagaaaccaggacaatctcctaaactactgatttactcggcatcctaccggtacactggagtccctgatcgcttcactggcagtggatctgggacggatttcactttcaccatcagcagtgtgaaggctgaagacctggcagtttattactgtcagcaacattatattactccgtggacgttcggtggaggcaccaagctggaaataaaa

SEQ ID NO: 8 - protein, 6 aa, synthetic construct
QHVSTA

SEQ ID NO: 9 - skipped

SEQ ID NO: 10 - protein, 9 aa, synthetic construct
QQHYITPWT

SEQ ID NO: 11 - protein, 121 aa, synthetic construct
DVQLQESGPGLVKPSQTLSLTCTVSGHSFTSDYAWNWIRQFPGKGLEWIGYISYSDSTNYNPSLKSRITISRDTSKNQFFLQLNSVTAADTATYYCARLDYGNYGGAMDYWGQGTSVTVSS

SEQ ID NO: 12 - DNA, 363 bp, synthetic construct
  source 1..363: mol_type = other DNA
gatgtgcagctgcaggagagcggccccggactggtgaagccttcccagaccctgtctctgacctgtacagtgtctggccacagcttcacatccgactacgcctggaactggatcaggcagtttccaggcaagggcctggagtggatcggctacatctcttatagcgactccaccaactataatccctctctgaagagccggatcaccatcagcagagatacatccaagaaccagttctttctgcagctgaacagcgtgacagccgccgacaccgccacatactattgcgcccggctggactacggcaattatggcggagccatggattactggggccagggcacctccgtgacagtgagctcc

SEQ ID NO: 13 - protein, 121 aa, synthetic construct
DVQLQESGPGLVKPSQTLSLTCTVSGHSFTSDYAWSWIRQPPGKGLEWIGYISYSDSTNYNPSLKSRVTISRDTSKNQFSLKLSSVTAADTAVYYCARLDYGNYGGAMDYWGQGTSVTVSS

SEQ ID NO: 14 - DNA, 363 bp, synthetic construct
  source 1..363: mol_type = other DNA
gatgtgcagctgcaggagtctggcccaggactggtgaagccaagccagaccctgtccctgacctgtacagtgtccggccactcttttacaagcgactacgcctggtcttggatcaggcagccccctggcaagggactggagtggatcggctacatctcctattctgacagcaccaactataatccctccctgaagtctcgggtgaccatctctagagatacaagcaagaaccagttctccctgaagctgagctccgtgaccgcagcagacacagccgtgtactattgcgcccggctggactacggcaattatggcggagccatggattactggggccagggcaccagcgtgacagtgtctagc

SEQ ID NO: 15 - protein, 121 aa, synthetic construct
DVQLQESGPGLVKPSQTLSLTCTVSGHSFTSDYAWSWIRQPPGKGLEWIGYISYSDSTNYNPSLKSRVTISVDTSKNQFSLKLSSVTAADTAVYYCARLDYGNYGGAMDYWGQGTSVTVSS

SEQ ID NO: 16 - DNA, 363 bp, synthetic construct
  source 1..363: mol_type = other DNA
gatgtgcagctgcaggagtctggcccaggactggtgaagccaagccagaccctgtccctgacctgtacagtgtccggccactcttttacaagcgactacgcctggtcttggatcagacagccccctggcaagggactggagtggatcggctacatctcctattctgacagcaccaactataatccctccctgaagtctagagtgaccatctctgtggatacaagcaagaaccagttctccctgaagctgagctccgtgaccgcagcagacacagccgtgtactattgcgcccggctggactacggcaattatggcggagccatggattactggggccagggcaccagcgtgacagtgtctagc

SEQ ID NO: 17 - protein, 121 aa, synthetic construct
DVQLQESGPGLVKPSQTLSLTCTVSGHSFTSDYAWNWIRQFPGKGLEWMGYISYSDSTNYNPSLKSRITISRDTSKNQFFLQLNSVTAADTATYYCARLDYGNYGGAMDYWGQGTSVTVSS

SEQ ID NO: 18 - DNA, 363 bp, synthetic construct
  source 1..363: mol_type = other DNA
gatgtgcagctgcaggagagcggccccggactggtgaagccttcccagaccctgtctctgacctgtacagtgtctggccacagcttcacatccgactacgcctggaactggatcaggcagtttccaggcaagggcctggagtggatgggctacatctcttatagcgactccaccaactataatccctctctgaagagccggatcaccatcagcagagatacatccaagaaccagttctttctgcagctgaacagcgtgacagccgccgacaccgccacatactattgcgcccggctggactacggcaattatggcggagccatggattactggggccagggcacctccgtgacagtgagctcc

SEQ ID NO: 19 - protein, 107 aa, synthetic construct
DIQMTQSPKSLSTSVGDRVTITCRSSQHVSTAVAWYQQKPGKSPKLLIYSASYRYSGVPDRFSGSGSGTDFTFTISSVQPEDFATYYCQQHYITPWTFGGGTKLEIK

SEQ ID NO: 20 - DNA, 321 bp, synthetic construct
  source 1..321: mol_type = other DNA
gacatccagatgacccagtcccctaagtccctgtctacaagcgtgggcgatcgggtgaccatcacatgtagaagctcccagcacgtgtctaccgcagtggcatggtaccagcagaagccaggcaagagccctaagctgctgatctattccgcctcttacaggtattccggagtgccagaccggtttagcggctccggctctggcaccgatttcacctttacaatctctagcgtgcagccagaggacttcgccacatactattgccagcagcactacatcaccccatggaccttcggcggcggcacaaagctggagatcaag

SEQ ID NO: 21 - protein, 107 aa, synthetic construct
DIQMTQSPSSLSASVGDRVTITCRSSQHVSTALAWYQQKPGKSPKLLIYSASSRYSGVPDRFSGSGSGTDFTFTISSLQPEDFATYYCQQHYITPWTFGGGTKLEIK

SEQ ID NO: 22 - DNA, 321 bp, synthetic construct
  source 1..321: mol_type = other DNA
gacatccagatgacccagtcccctagctccctgtctgccagcgtgggcgatagggtgaccatcacatgtagatctagccagcacgtgtctacagccctggcatggtaccagcagaagccaggcaagagccctaagctgctgatctactccgcctcctctaggtattctggagtgccagaccggttttccggctctggcagcggcaccgatttcacctttacaatcagctccctgcagccagaggacttcgccacatactattgccagcagcactatatcaccccatggaccttcggcggcggcaccaagctggagatcaag

SEQ ID NO: 23 - protein, 107 aa, synthetic construct
DIQMTQSPSSLSASVGDRVTITCRASQHVSTALAWYQQKPGKAPKLLIYSASSLQSGVPSRFSGSGSGTDFTLTISSLQPEDFATYYCQQHYITPWTFGGGTKLEIK

SEQ ID NO: 24 - DNA, 321 bp, synthetic construct
  source 1..321: mol_type = other DNA
gacatccagatgacccagtcccctagctccctgagcgcctccgtgggcgatagggtgaccatcacatgtagagcctctcagcacgtgagcacagccctggcatggtaccagcagaagccaggcaaggcccctaagctgctgatctatagcgcctctagcctgcagtccggagtgccatctcggttctctggcagcggctccggaaccgactttaccctgacaatctcctctctgcagccagaggatttcgccacatactattgccagcagcactacatcaccccatggaccttcggcggcggcaccaagctggagatcaag

SEQ ID NO: 25 - protein, 107 aa, synthetic construct
DIQMTQSPKSMSTSVGDRVTITCRSSQHVSTAVAWYQQKPGKSPKLLIYSASYRYSGVPDRFSGSGSGTDFTFTISSVQPEDFATYYCQQHYITPWTFGGGTKLEIK

SEQ ID NO: 26 - DNA, 321 bp, synthetic construct
  source 1..321: mol_type = other DNA
gacatccagatgacccagtcccctaagtccatgtctacaagcgtgggcgacagggtgaccatcacatgtagaagctcccagcacgtgtctaccgcagtggcatggtaccagcagaagccaggcaagagccctaagctgctgatctattccgcctcttacaggtattccggagtgccagaccggtttagcggctccggctctggcaccgatttcacctttacaatctctagcgtgcagccagaggacttcgccacatactattgccagcagcactacatcaccccatggaccttcggcggcggcacaaagctggagatcaag

SEQ ID NO: 27 - protein, 118 aa, synthetic construct
EVKLVESGGGLVKPGGSLKLSCAASGFAFSSYDMSWVRQTPEKRLEWVATISGGGRYTYYPDSVKGRFTISRDNARNTLYLQMSSLRSEDTALYYCANRYGEAWFAYWGQGTLVTVSA

SEQ ID NO: 28 - protein, 107 aa, synthetic construct
DIKMTQSPSSMYASLGERVTFTCKASQDINTYLSWFQQKPGKSPKTLIYRANRLVDGVPSRFSGSGSGQDYSLTISSLEYEDMGIYYCLQYDEFPLTFGAGTKLELK

SEQ ID NO: 29 - protein, 8 aa, synthetic construct
GFAFSSYD

SEQ ID NO: 30 - protein, 8 aa, synthetic construct
ISGGGRYT

SEQ ID NO: 31 - protein, 11 aa, synthetic construct
ANRYGEAWFAY

SEQ ID NO: 32 - protein, 6 aa, synthetic construct
QDINTY

SEQ ID NO: 33 - skipped

SEQ ID NO: 34 - protein, 9 aa, synthetic construct
LQYDEFPLT

SEQ ID NO: 35 - protein, 124 aa, synthetic construct
QVKLQESGPELVKPGASMKISCKASGYSFTGYTMNWVKQSHGKNLEWIGLINPYNNITNYNQKFMGKATFTVDKSSSTAYMELLRLTSEDSGVYFCARLDYRSYWGQGTLVTVSAAKTTPPSVY

SEQ ID NO: 36 - protein, 126 aa, synthetic construct
QAVVTQESALTTSPGETVTLTCRSSTGAVTTSNFANWVQEKPDHLFTSLIGGTNNRAPGVPARFSGSLIGDKAALTITGAQTEDEAIYFCALWYSNHWVFGGGTKLTVLGQPKSSPSVTLFQGQFC

SEQ ID NO: 37 - protein, 8 aa, synthetic construct
GYSFTGYT

SEQ ID NO: 38 - protein, 8 aa, synthetic construct
INPYNNIT

SEQ ID NO: 39 - protein, 8 aa, synthetic construct
ARLDYRSY

SEQ ID NO: 40 - protein, 9 aa, synthetic construct
TGAVTTSNF

SEQ ID NO: 41 - skipped

SEQ ID NO: 42 - protein, 9 aa, synthetic construct
ALWYSNHWV

SEQ ID NO: 43 - protein, 118 aa, synthetic construct
EVQLVESGGGLVQPGGSLRLSCAASGFAFSSYDMSWVRQAPGKGLDWVATISGGGRYTYYPDSVKGRFTISRDNSKNNLYLQMNSLRAEDTALYYCANRYGEAWFAYWGQGTLVTVSS

SEQ ID NO: 44 - protein, 107 aa, synthetic construct
DIQMTQSPSSMSASVGDRVTFTCRASQDINTYLSWFQQKPGKSPKTLIYRANRLVSGVPSRFSGSGSGQDYTLTISSLQPEDMATYYCLQYDEFPLTFGAGTKLELK

SEQ ID NO: 45 - protein, 115 aa, synthetic construct
QVQLVESGAELVKPGASMKISCKASGYSFTGYTMNWVKQAPGQGLEWIGLINPYNNITNYNQKFMGKATFTVDKSISTAYMELSRLTSDDSGVYFCARLDYRSYWGQGTLVTVSA

SEQ ID NO: 46 - protein, 115 aa, synthetic construct
QVQLVESGAEVKKPGASVKVSCKASGYSFTGYTMNWVRQAPGQGLEWIGLINPYNNITNYAQKFQGRVTFTVDTSISTAYMELSRLRSDDTGVYFCARLDYRSYWGQGTLVTVSA

SEQ ID NO: 47 - protein, 115 aa, synthetic construct
QVQLVESGAELVKPGASMKISCKASGYSFTGYTMNWVKQAPGQCLEWIGLINPYNNITNYNQKFMGKATFTVDKSISTAYMELSRLTSDDSGVYFCARLDYRSYWGQGTLVTVSA

SEQ ID NO: 48 - protein, 115 aa, synthetic construct
QVQLVESGAEVKKPGASVKVSCKASGYSFTGYTMNWVRQAPGQCLEWIGLINPYNNITNYAQKFQGRVTFTVDTSISTAYMELSRLRSDDTGVYFCARLDYRSYWGQGTLVTVSA

SEQ ID NO: 49 - protein, 109 aa, synthetic construct
QAVVTQEPSLTVSPGGTVTLTCGSSTGAVTTSNFANWVQEKPGQAFRSLIGGTNNRASWVPARFSGSLLGGKAALTISGAQPEDEAEYFCALWYSNHWVFGGGTKLTVL

SEQ ID NO: 50 - protein, 109 aa, synthetic construct
QAVVTQEPSLTVSPGGTVTLTCGSSTGAVTTSNFPNWVQQKPGQAPRSLIGGTNNKASWTPARFSGSLLGGKAALTISGAQPEDEAEYYCALWYSNHWVFGGGTKLTVL

SEQ ID NO: 51 - protein, 110 aa, synthetic construct
QAVVTQEPSLTVSPGGTVTLTCGSSTGAVTTSNFANWVQEKPGQAFRSLIGGTNNRASWVPARFSGSLLGGKAALTISGAQPEDEAEYFCALWYSNHWVFGCGTKLTVLR

SEQ ID NO: 52 - protein, 110 aa, synthetic construct
QAVVTQEPSLTVSPGGTVTLTCGSSTGAVTTSNFPNWVQQKPGQAPRSLIGGTNNKASWTPARFSGSLLGGKAALTISGAQPEDEAEYYCALWYSNHWVFGCGTKLTVLR

SEQ ID NO: 53 - protein, 448 aa, synthetic construct
EVQLVESGGGLVQPGGSLRLSCAASGFAFSSYDMSWVRQAPGKGLDWVATISGGGRYTYYPDSVKGRFTISRDNSKNNLYLQMNSLRAEDTALYYCANRYGEAWFAYWGQGTLVTVSSASTKGPSVFPLAPSSKSTSGGTAALGCLVKDYFPEPVTVSWNSGALTSGVHTFPAVLQSSGLYSLSSVVTVPSSSLGTQTYICNVNHKPSNTKVDKKVEPKSCDKTHTCPPCPAPEAAGAPSVFLFPPKPKDTLMISRTPEVTCVVVDVSHEDPEVKFNWYVDGVEVHNAKTKPREEQYNSTYRVVSVLTVLHQDWLNGKEYKCKVSNKALPAPIEKTISKAKGQPREPQVYTLPPSRDELTKNQVSLTCLVKGFYPSDIAVEWESNGQPENNYKTTPPVLDSDGSFFLYSKLTVDKSRWQQGNVFSCSVMHEALHNHYTQKSLSLSPGK

SEQ ID NO: 54 - protein, 214 aa, synthetic construct
DIQMTQSPSSMSASVGDRVTFTCRASQDINTYLSWFQQKPGKSPKTLIYRANRLVSGVPSRFSGSGSGQDYTLTISSLQPEDMATYYCLQYDEFPLTFGAGTKLELKRTVAAPSVFIFPPSDEQLKSGTASVVCLLNNFYPREAKVQWKVDNALQSGNSQESVTEQDSKDSTYSLSSTLTLSKADYEKHKVYACEVTHQGLSSPVTKSFNRGEC

SEQ ID NO: 55 - protein, 15 aa, synthetic construct
GGGGSGGGGSGGGGS

SEQ ID NO: 56 - protein, 20 aa, synthetic construct
GGGGSGGGGSGGGGSGGGGS

SEQ ID NO: 57 - protein, 713 aa, synthetic construct
EVQLVESGGGLVQPGGSLRLSCAASGFAFSSYDMSWVRQAPGKGLDWVATISGGGRYTYYPDSVKGRFTISRDNSKNNLYLQMNSLRAEDTALYYCANRYGEAWFAYWGQGTLVTVSSASTKGPSVFPLAPSSKSTSGGTAALGCLVKDYFPEPVTVSWNSGALTSGVHTFPAVLQSSGLYSLSSVVTVPSSSLGTQTYICNVNHKPSNTKVDKKVEPKSCDKTHTCPPCPAPEAAGAPSVFLFPPKPKDTLMISRTPEVTCVVVDVSHEDPEVKFNWYVDGVEVHNAKTKPREEQYNSTYRVVSVLTVLHQDWLNGKEYKCKVSNKALPAPIEKTISKAKGQPREPQVYTLPPSRDELTKNQVSLTCLVKGFYPSDIAVEWESNGQPENNYKTTPPVLDSDGSFFLYSKLTVDKSRWQQGNVFSCSVMHEALHNHYTQKSLSLSPGKGGGGSGGGGSGGGGSGGGGSQVQLVESGAEVKKPGASVKVSCKASGYSFTGYTMNWVRQAPGQCLEWIGLINPYNNITNYAQKFQGRVTFTVDTSISTAYMELSRLRSDDTGVYFCARLDYRSYWGQGTLVTVSAGGGGSGGGGSGGGGSGGGGSQAVVTQEPSLTVSPGGTVTLTCGSSTGAVTTSNFPNWVQQKPGQAPRSLIGGTNNKASWTPARFSGSLLGGKAALTISGAQPEDEAEYYCALWYSNHWVFGCGTKLTVLR

SEQ ID NO: 58 - DNA, 2139 bp, synthetic construct
  source 1..2139: mol_type = other DNA
gaagtgcagctggtcgagtctgggggagggctggtgcagcccggcgggtcactgcgactgagctgcgcagcttccggattcgcctttagctcctacgacatgtcctgggtgcgacaggcaccaggaaagggactggattgggtcgctactatctcaggaggcgggagatacacctactatcctgacagcgtcaagggccggttcacaatctctagagataacagtaagaacaatctgtatctgcagatgaacagcctgagggctgaggacaccgcactgtactattgtgccaaccgctacggggaagcatggtttgcctattgggggcagggaaccctggtgacagtctctagtgccagcaccaaagggcccagcgtgtttcctctcgccccctcctccaaaagcaccagcggaggaaccgctgctctcggatgtctggtgaaggactacttccctgaacccgtcaccgtgagctggaatagcggcgctctgacaagcggagtccatacattccctgctgtgctgcaaagcagcggactctattccctgtccagcgtcgtcacagtgcccagcagcagcctgggcacccagacctacatctgtaacgtcaaccacaagccctccaacaccaaggtggacaagaaagtggagcccaaatcctgcgacaagacacacacctgtcccccctgtcctgctcccgaagctgctggagcccctagcgtcttcctctttcctcccaaacccaaggacaccctcatgatcagcagaacccctgaagtcacctgtgtcgtcgtggatgtcagccatgaggaccccgaggtgaaattcaactggtatgtcgatggcgtcgaggtgcacaacgccaaaaccaagcccagggaggaacagtacaactccacctacagggtggtgtccgtgctgacagtcctccaccaggactggctgaacggcaaggagtacaagtgcaaggtgtccaacaaggctctccctgcccccattgagaagaccatcagcaaggccaaaggccaacccagggagccccaggtctatacactgcctccctccagggacgaactcaccaagaaccaggtgtccctgacctgcctggtcaagggcttttatcccagcgacatcgccgtcgagtgggagtccaacggacagcccgagaataactacaagaccacccctcctgtcctcgactccgacggctccttcttcctgtacagcaaactgaccgtggataagtccagatggcagcagggcaatgtcttttcatgttccgtgatgcacgaggcactgcacaaccactatacccagaagtctctgagtctgtcaccaggaaaaggaggaggaggctctggaggaggcggaagtggaggcggaggatcaggagggggaggatctcaggtgcagctggtcgaatccggagccgaggtgaagaaacccggcgcttccgtgaaggtctcttgcaaagcatcaggctacagcttcacagggtatactatgaactgggtgcggcaggcacctggacagtgtctggaatggatcggcctgattaacccatacaacaacatcactaactacgcccagaagttccagggccgggtgacttttaccgtggacactagcatttccaccgcttacatggagctgagtcggctgagatcagacgataccggcgtgtatttttgcgcaaggctggattacagaagttattggggacagggaacacttgttacagtctctgctggaggaggcggatctggaggaggaggatctggcggaggaggcagtggaggaggaggatcacaggctgtggttactcaggaaccaagcctgaccgtgagccccggaggcacagtcactctgacctgtgggagctccacaggagctgtgaccacatctaacttccctaattgggtgcagcagaagccaggacaggcacctcgatccctgatcgggggaaccaacaacaaggccagctggacacccgccagattttctggcagtctgctgggcgggaaagccgctctgaccattagcggcgctcagcctgaggacgaagcagagtactattgcgccctgtggtatagtaatcattgggtgttcgggtgtgggacaaaactgaccgtgctgaga

SEQ ID NO: 59 - protein, 214 aa, synthetic construct; identical to SEQ ID NO: 54

SEQ ID NO: 60 - DNA, 642 bp, synthetic construct
  source 1..642: mol_type = other DNA
gacattcagatgactcagagcccctcctccatgtccgcctctgtgggcgacagggtcaccttcacatgccgcgctagtcaggatatcaacacctacctgagctggtttcagcagaagccagggaaaagccccaagacactgatctaccgggctaatagactggtgtctggagtcccaagtcggttcagtggctcagggagcggacaggactacactctgaccatcagctccctgcagcctgaggacatggcaacctactattgcctgcagtatgatgagttcccactgacctttggcgccgggacaaaactggagctgaagcgaactgtggccgctccctccgtcttcatttttcccccttctgacgaacagctgaaatcaggcacagccagcgtggtctgtctgctgaacaatttctaccctagagaggcaaaagtgcagtggaaggtcgataacgccctgcagtccggcaacagccaggagagtgtgactgaacaggactcaaaagatagcacctattccctgtctagtacactgactctgtccaaggctgattacgagaagcacaaagtgtatgcatgcgaagtgacacatcagggactgtcaagccccgtgactaagtcttttaaccggggcgaatgt

SEQ ID NO: 61 - protein, 8 aa, synthetic construct
GFAFSSYD

SEQ ID NO: 62 - protein, 8 aa, synthetic construct
ISGGGRYT

SEQ ID NO: 63 - protein, 11 aa, synthetic construct
ANRYGEAWFAY

SEQ ID NO: 64 - protein, 8 aa, synthetic construct
GYSFTGYT

SEQ ID NO: 65 - protein, 8 aa, synthetic construct
INPYNNIT

SEQ ID NO: 66 - protein, 8 aa, synthetic construct
ARLDYRSY

SEQ ID NO: 67 - protein, 9 aa, synthetic construct
TGAVTTSNF

SEQ ID NO: 68 - skipped

SEQ ID NO: 69 - protein, 9 aa, synthetic construct
ALWYSNHWV

SEQ ID NO: 70 - protein, 6 aa, synthetic construct
QDINTY

SEQ ID NO: 71 - skipped

SEQ ID NO: 72 - protein, 9 aa, synthetic construct
LQYDEFPLT

SEQ ID NO: 73 - protein, 118 aa, synthetic construct; identical to SEQ ID NO: 43

SEQ ID NO: 74 - protein, 115 aa, synthetic construct; identical to SEQ ID NO: 48

SEQ ID NO: 75 - protein, 110 aa, synthetic construct; identical to SEQ ID NO: 52

SEQ ID NO: 76 - protein, 107 aa, synthetic construct; identical to SEQ ID NO: 44

SEQ ID NO: 77 - protein, 232 aa, synthetic construct
PRGPTIKPCPPCKCPAPNLLGGPSVFIFPPKIKDVLMISLSPIVTCVVVDVSEDDPDVQISWFVNNVEVHTAQTQTHREDYNSTLRVVSALPIQHQDWMSGKEFKCKVNNKDLPAPIERTISKPKGSVRAPQVYVLPPPEEEMTKKQVTLTCMVTDFMPEDIYVEWTNNGKTELNYKNTEPVLDSDGSYFMYSKLRVEKKNWVERNSYSCSVVHEGLHNHHTTKSFSRTPGK

SEQ ID NO: 78 - protein, 225 aa, synthetic construct
THTCPPCPAPELLGGPSVFLFPPKPKDTLMISRTPEVTCVVVDVSHEDPEVKFNWYVDGVEVHNAKTKPREEQYNSTYRVVSVLTVLHQDWLNGKEYKCKVSNKALPAPIEKTISKAKGQPREPQVYTLPPSRDELTKNQVSLTCLVKGFYPSDIAVEWESNGQPENNYKTTPPVLDSDGSFFLYSKLTVDKSRWQQGNVFSCSVMHEALHNHYTQKSLSLSPGK